European Patent Application EP 4 273 174 A1, published November 8, 2023. Title: HUMAN PAPILLOMAVIRUS TYPE 31 CHIMERIC PROTEIN AND USE THEREOF. Applicant: Institute of Basic Medical Sciences, Chinese Academy of Medical Sciences. The sequence listing filed with the application follows.

SEQUENCE LISTING (60 sequences)

SEQ ID NO: 1 - protein, 504 aa, HPV31
MSLWRPSEATVYLPPVPVSKVVSTDEYVTRTNIYYHAGSARLLTVGHPYYSIPKSDNPKKIVVPKVSGLQYRVFRVRLPDPNKFGFPDTSFYNPETQRLVWACVGLEVGRGQPLGVGISGHPLLNKFDDTENSNRYAGGPGTDNRECISMDYKQTQLCLLGCKPPIGEHWGKGSPCSNNAITPGDCPPLELKNSVIQDGDMVDTGFGAMDFTALQDTKSNVPLDICNSICKYPDYLKMVAEPYGDTLFFYLRREQMFVRHFFNRSGTVGESVPTDLYIKGSGSTATLANSTYFPTPSGSMVTSDAQIFNKPYWMQRAQGHNNGICWGNQLFVTVVDTTRSTNMSVCAAIANSDTTFKSSNFKEYLRHGEEFDLQFIFQLCKITLSADIMTYIHSMNPAILEDWNFGLTTPPSGSLEDTYRFVTSQAITCQKTAPQKPKEDPFKDYVFWEVNLKEKFSADLDQFPLGRKFLLQAGYRARPKFKAGKRSAPSASTTTPAKRKKTKK

SEQ ID NO: 2 - protein, 475 aa, HPV73
MRRKRDTHIRKKRASATQLYKTCKQAGTCPPDVIPKVEGSTIADNILKYGSIGVFFGGLGIGSGSGSGGRTGYVPLSTGTPSKPVEMPLQPIRPSVVTSVGPSDSSIVSLVEESSFIESGIPGPTSIVPSTSGFDITTSVNSTPAIIDVSAISDTTQISVTTFKNPTFTDPSVLQPPPPLEASGRLLFSNDTVTTHSYENIPLDTFVVTTDHNSIVSSTPIPGRQPAARLGLYGRAIQQVKVVDPAFLTTPTRLVTYDNPAFEGLQDTTLEFQHSDLHNAPDSDFLDIVKLHRPALTSRKTGIRVSRLGQRATLSTRSGKRIGAKVHFYHDISPIPTNDIEMQPLVTPQTPSIVTGSSINDGLYDVFLENDVEDTVVQQTYTPTSIHSNSLVSSDVSTATANTTIPFSTGLDTHPGPDIALPLPSTETIFTPIVPLQPAGPIYIYGSGFILHPSYYLLKRKRKRLSYSFTDVATY

SEQ ID NO: 3 - protein, 504 aa, Artificial Sequence
  VARIANT (274)..(274): T274N
MSLWRPSEATVYLPPVPVSKVVSTDEYVTRTNIYYHAGSARLLTVGHPYYSIPKSDNPKKIVVPKVSGLQYRVFRVRLPDPNKFGFPDTSFYNPETQRLVWACVGLEVGRGQPLGVGISGHPLLNKFDDTENSNRYAGGPGTDNRECISMDYKQTQLCLLGCKPPIGEHWGKGSPCSNNAITPGDCPPLELKNSVIQDGDMVDTGFGAMDFTALQDTKSNVPLDICNSICKYPDYLKMVAEPYGDTLFFYLRREQMFVRHFFNRSGTVGESVPNDLYIKGSGSTATLANSTYFPTPSGSMVTSDAQIFNKPYWMQRAQGHNNGICWGNQLFVTVVDTTRSTNMSVCAAIANSDTTFKSSNFKEYLRHGEEFDLQFIFQLCKITLSADIMTYIHSMNPAILEDWNFGLTTPPSGSLEDTYRFVTSQAITCQKTAPQKPKEDPFKDYVFWEVNLKEKFSADLDQFPLGRKFLLQAGYRARPKFKAGKRSAPSASTTTPAKRKKTKK

SEQ ID NO: 4 - protein, 501 aa, Artificial Sequence
  VARIANT (274)..(274): T274N delta N4
MRPSEATVYLPPVPVSKVVSTDEYVTRTNIYYHAGSARLLTVGHPYYSIPKSDNPKKIVVPKVSGLQYRVFRVRLPDPNKFGFPDTSFYNPETQRLVWACVGLEVGRGQPLGVGISGHPLLNKFDDTENSNRYAGGPGTDNRECISMDYKQTQLCLLGCKPPIGEHWGKGSPCSNNAITPGDCPPLELKNSVIQDGDMVDTGFGAMDFTALQDTKSNVPLDICNSICKYPDYLKMVAEPYGDTLFFYLRREQMFVRHFFNRSGTVGESVPNDLYIKGSGSTATLANSTYFPTPSGSMVTSDAQIFNKPYWMQRAQGHNNGICWGNQLFVTVVDTTRSTNMSVCAAIANSDTTFKSSNFKEYLRHGEEFDLQFIFQLCKITLSADIMTYIHSMNPAILEDWNFGLTTPPSGSLEDTYRFVTSQAITCQKTAPQKPKEDPFKDYVFWEVNLKEKFSADLDQFPLGRKFLLQAGYRARPKFKAGKRSAPSASTTTPAKRKKTKK

SEQ ID NO: 5 - protein, 475 aa, Artificial Sequence
  VARIANT (1)..(475): 31L1 delta C29
MSLWRPSEATVYLPPVPVSKVVSTDEYVTRTNIYYHAGSARLLTVGHPYYSIPKSDNPKKIVVPKVSGLQYRVFRVRLPDPNKFGFPDTSFYNPETQRLVWACVGLEVGRGQPLGVGISGHPLLNKFDDTENSNRYAGGPGTDNRECISMDYKQTQLCLLGCKPPIGEHWGKGSPCSNNAITPGDCPPLELKNSVIQDGDMVDTGFGAMDFTALQDTKSNVPLDICNSICKYPDYLKMVAEPYGDTLFFYLRREQMFVRHFFNRSGTVGESVPTDLYIKGSGSTATLANSTYFPTPSGSMVTSDAQIFNKPYWMQRAQGHNNGICWGNQLFVTVVDTTRSTNMSVCAAIANSDTTFKSSNFKEYLRHGEEFDLQFIFQLCKITLSADIMTYIHSMNPAILEDWNFGLTTPPSGSLEDTYRFVTSQAITCQKTAPQKPKEDPFKDYVFWEVNLKEKFSADLDQFPLGRKFLLQAGY

SEQ ID NO: 6 - protein, 475 aa, Artificial Sequence
  VARIANT (1)..(475): T274N delta C29
MSLWRPSEATVYLPPVPVSKVVSTDEYVTRTNIYYHAGSARLLTVGHPYYSIPKSDNPKKIVVPKVSGLQYRVFRVRLPDPNKFGFPDTSFYNPETQRLVWACVGLEVGRGQPLGVGISGHPLLNKFDDTENSNRYAGGPGTDNRECISMDYKQTQLCLLGCKPPIGEHWGKGSPCSNNAITPGDCPPLELKNSVIQDGDMVDTGFGAMDFTALQDTKSNVPLDICNSICKYPDYLKMVAEPYGDTLFFYLRREQMFVRHFFNRSGTVGESVPNDLYIKGSGSTATLANSTYFPTPSGSMVTSDAQIFNKPYWMQRAQGHNNGICWGNQLFVTVVDTTRSTNMSVCAAIANSDTTFKSSNFKEYLRHGEEFDLQFIFQLCKITLSADIMTYIHSMNPAILEDWNFGLTTPPSGSLEDTYRFVTSQAITCQKTAPQKPKEDPFKDYVFWEVNLKEKFSADLDQFPLGRKFLLQAGY

SEQ ID NO: 7 - protein, 474 aa, Artificial Sequence
  VARIANT (1)..(474): T274N delta N2C29
MLWRPSEATVYLPPVPVSKVVSTDEYVTRTNIYYHAGSARLLTVGHPYYSIPKSDNPKKIVVPKVSGLQYRVFRVRLPDPNKFGFPDTSFYNPETQRLVWACVGLEVGRGQPLGVGISGHPLLNKFDDTENSNRYAGGPGTDNRECISMDYKQTQLCLLGCKPPIGEHWGKGSPCSNNAITPGDCPPLELKNSVIQDGDMVDTGFGAMDFTALQDTKSNVPLDICNSICKYPDYLKMVAEPYGDTLFFYLRREQMFVRHFFNRSGTVGESVPNDLYIKGSGSTATLANSTYFPTPSGSMVTSDAQIFNKPYWMQRAQGHNNGICWGNQLFVTVVDTTRSTNMSVCAAIANSDTTFKSSNFKEYLRHGEEFDLQFIFQLCKITLSADIMTYIHSMNPAILEDWNFGLTTPPSGSLEDTYRFVTSQAITCQKTAPQKPKEDPFKDYVFWEVNLKEKFSADLDQFPLGRKFLLQAGY

SEQ ID NO: 8 - protein, 472 aa, Artificial Sequence
  VARIANT (1)..(472): T274N delta N4C29
MRPSEATVYLPPVPVSKVVSTDEYVTRTNIYYHAGSARLLTVGHPYYSIPKSDNPKKIVVPKVSGLQYRVFRVRLPDPNKFGFPDTSFYNPETQRLVWACVGLEVGRGQPLGVGISGHPLLNKFDDTENSNRYAGGPGTDNRECISMDYKQTQLCLLGCKPPIGEHWGKGSPCSNNAITPGDCPPLELKNSVIQDGDMVDTGFGAMDFTALQDTKSNVPLDICNSICKYPDYLKMVAEPYGDTLFFYLRREQMFVRHFFNRSGTVGESVPNDLYIKGSGSTATLANSTYFPTPSGSMVTSDAQIFNKPYWMQRAQGHNNGICWGNQLFVTVVDTTRSTNMSVCAAIANSDTTFKSSNFKEYLRHGEEFDLQFIFQLCKITLSADIMTYIHSMNPAILEDWNFGLTTPPSGSLEDTYRFVTSQAITCQKTAPQKPKEDPFKDYVFWEVNLKEKFSADLDQFPLGRKFLLQAGY

SEQ ID NO: 9 - protein, 471 aa, Artificial Sequence
  VARIANT (1)..(471): T274N delta N5C29
MPSEATVYLPPVPVSKVVSTDEYVTRTNIYYHAGSARLLTVGHPYYSIPKSDNPKKIVVPKVSGLQYRVFRVRLPDPNKFGFPDTSFYNPETQRLVWACVGLEVGRGQPLGVGISGHPLLNKFDDTENSNRYAGGPGTDNRECISMDYKQTQLCLLGCKPPIGEHWGKGSPCSNNAITPGDCPPLELKNSVIQDGDMVDTGFGAMDFTALQDTKSNVPLDICNSICKYPDYLKMVAEPYGDTLFFYLRREQMFVRHFFNRSGTVGESVPNDLYIKGSGSTATLANSTYFPTPSGSMVTSDAQIFNKPYWMQRAQGHNNGICWGNQLFVTVVDTTRSTNMSVCAAIANSDTTFKSSNFKEYLRHGEEFDLQFIFQLCKITLSADIMTYIHSMNPAILEDWNFGLTTPPSGSLEDTYRFVTSQAITCQKTAPQKPKEDPFKDYVFWEVNLKEKFSADLDQFPLGRKFLLQAGY

SEQ ID NO: 10 - protein, 468 aa, Artificial Sequence
  VARIANT (1)..(468): T274N delta N8C29
MATVYLPPVPVSKVVSTDEYVTRTNIYYHAGSARLLTVGHPYYSIPKSDNPKKIVVPKVSGLQYRVFRVRLPDPNKFGFPDTSFYNPETQRLVWACVGLEVGRGQPLGVGISGHPLLNKFDDTENSNRYAGGPGTDNRECISMDYKQTQLCLLGCKPPIGEHWGKGSPCSNNAITPGDCPPLELKNSVIQDGDMVDTGFGAMDFTALQDTKSNVPLDICNSICKYPDYLKMVAEPYGDTLFFYLRREQMFVRHFFNRSGTVGESVPNDLYIKGSGSTATLANSTYFPTPSGSMVTSDAQIFNKPYWMQRAQGHNNGICWGNQLFVTVVDTTRSTNMSVCAAIANSDTTFKSSNFKEYLRHGEEFDLQFIFQLCKITLSADIMTYIHSMNPAILEDWNFGLTTPPSGSLEDTYRFVTSQAITCQKTAPQKPKEDPFKDYVFWEVNLKEKFSADLDQFPLGRKFLLQAGY

SEQ ID NO: 11 - protein, 466 aa, Artificial Sequence
  VARIANT (1)..(466): T274N delta N10C29
MVYLPPVPVSKVVSTDEYVTRTNIYYHAGSARLLTVGHPYYSIPKSDNPKKIVVPKVSGLQYRVFRVRLPDPNKFGFPDTSFYNPETQRLVWACVGLEVGRGQPLGVGISGHPLLNKFDDTENSNRYAGGPGTDNRECISMDYKQTQLCLLGCKPPIGEHWGKGSPCSNNAITPGDCPPLELKNSVIQDGDMVDTGFGAMDFTALQDTKSNVPLDICNSICKYPDYLKMVAEPYGDTLFFYLRREQMFVRHFFNRSGTVGESVPNDLYIKGSGSTATLANSTYFPTPSGSMVTSDAQIFNKPYWMQRAQGHNNGICWGNQLFVTVVDTTRSTNMSVCAAIANSDTTFKSSNFKEYLRHGEEFDLQFIFQLCKITLSADIMTYIHSMNPAILEDWNFGLTTPPSGSLEDTYRFVTSQAITCQKTAPQKPKEDPFKDYVFWEVNLKEKFSADLDQFPLGRKFLLQAGY

SEQ ID NO: 12 - protein, 501 aa, Artificial Sequence
  VARIANT (1)..(501): T274N-CS1
MRPSEATVYLPPVPVSKVVSTDEYVTRTNIYYHAGSARLLTVGHPYYSIPKSDNPKKIVVPKVSGLQYRVFRVRLPDPNKFGFPDTSFYNPETQRLVWACVGLEVGRGQPLGVGISGHPLLNKFDDTENSNRYAGGPGTDNRECISMDYKQTQLCLLGCKPPIGEHWGKGSPCSNNAITPGDCPPLELKNSVIQDGDMVDTGFGAMDFTALQDTKSNVPLDICNSICKYPDYLKMVAEPYGDTLFFYLRREQMFVRHFFNRSGTVGESVPNDLYIKGSGSTATLANSTYFPTPSGSMVTSDAQIFNKPYWMQRAQGHNNGICWGNQLFVTVVDTTRSTNMSVCAAIANSDTTFKSSNFKEYLRHGEEFDLQFIFQLCKITLSADIMTYIHSMNPAILEDWNFGLTTPPSGSLEDTYRFVTSQAITCQKTAPQKPKEDPFKDYVFWEVNLKEKFSADLDQFPLGRKFLLQAGYRAGPSFAAGAGSAPSASTTTPAGGSATGS

SEQ ID NO: 13 - protein, 501 aa, Artificial Sequence
  VARIANT (1)..(501): T274N-CS2
MRPSEATVYLPPVPVSKVVSTDEYVTRTNIYYHAGSARLLTVGHPYYSIPKSDNPKKIVVPKVSGLQYRVFRVRLPDPNKFGFPDTSFYNPETQRLVWACVGLEVGRGQPLGVGISGHPLLNKFDDTENSNRYAGGPGTDNRECISMDYKQTQLCLLGCKPPIGEHWGKGSPCSNNAITPGDCPPLELKNSVIQDGDMVDTGFGAMDFTALQDTKSNVPLDICNSICKYPDYLKMVAEPYGDTLFFYLRREQMFVRHFFNRSGTVGESVPNDLYIKGSGSTATLANSTYFPTPSGSMVTSDAQIFNKPYWMQRAQGHNNGICWGNQLFVTVVDTTRSTNMSVCAAIANSDTTFKSSNFKEYLRHGEEFDLQFIFQLCKITLSADIMTYIHSMNPAILEDWNFGLTTPPSGSLEDTYRFVTSQAITCQKTAPQKPKEDPFKDYVFWEVNLKEKFSADLDQFPLGRKFLLQAGYGAGPSFAAGAGSAPSASTTTPAGGSATGS

SEQ ID NO: 14 - protein, 501 aa, Artificial Sequence
  VARIANT (1)..(501): T274N-CS3
MRPSEATVYLPPVPVSKVVSTDEYVTRTNIYYHAGSARLLTVGHPYYSIPKSDNPKKIVVPKVSGLQYRVFRVRLPDPNKFGFPDTSFYNPETQRLVWACVGLEVGRGQPLGVGISGHPLLNKFDDTENSNRYAGGPGTDNRECISMDYKQTQLCLLGCKPPIGEHWGKGSPCSNNAITPGDCPPLELKNSVIQDGDMVDTGFGAMDFTALQDTKSNVPLDICNSICKYPDYLKMVAEPYGDTLFFYLRREQMFVRHFFNRSGTVGESVPNDLYIKGSGSTATLANSTYFPTPSGSMVTSDAQIFNKPYWMQRAQGHNNGICWGNQLFVTVVDTTRSTNMSVCAAIANSDTTFKSSNFKEYLRHGEEFDLQFIFQLCKITLSADIMTYIHSMNPAILEDWNFGLTTPPSGSLEDTYRFVTSQAITCQKTAPQKPKEDPFKDYVFWEVNLKEKFSADLDQFPLGRKFLLQAGYRAGPSFKAGAGSAPSASTTTPAGGSATGS

SEQ ID NO: 15 - protein, 21 aa, HPV73
QLYKTCKQAGTCPPDVIPKVE

SEQ ID NO: 16 - protein, 21 aa, HPV73
LYKTCKQAGTCPPDVIPKVEG

SEQ ID NO: 17 - protein, 17 aa, HPV73
LYKTCKQAGTCPPDVIP

SEQ ID NO: 18 - protein, 492 aa, Artificial Sequence
  PEPTIDE (1)..(492): 31L1DE132-136/dE
MRPSEATVYLPPVPVSKVVSTDEYVTRTNIYYHAGSARLLTVGHPYYSIPKSDNPKKIVVPKVSGLQYRVFRVRLPDPNKFGFPDTSFYNPETQRLVWACVGLEVGRGQPLGVGISGHPLLNKFDDTENSNRGPQLYKTCKQAGTCPPDVIPKVEGPGTDNRECISMDYKQTQLCLLGCKPPIGEHWGKGSPCSNNAITPGDCPPLELKNSVIQDGDMVDTGFGAMDFTALQDTKSNVPLDICNSICKYPDYLKMVAEPYGDTLFFYLRREQMFVRHFFNRSGTVGESVPNDLYIKGSGSTATLANSTYFPTPSGSMVTSDAQIFNKPYWMQRAQGHNNGICWGNQLFVTVVDTTRSTNMSVCAAIANSDTTFKSSNFKEYLRHGEEFDLQFIFQLCKITLSADIMTYIHSMNPAILEDWNFGLTTPPSGSLEDTYRFVTSQAITCQKTAPQKPKEDPFKDYVFWEVNLKEKFSADLDQFPLGRKFLLQAGY

SEQ ID NO: 19 - protein, 488 aa, Artificial Sequence
  PEPTIDE (1)..(488): 31L1DE132-136/dES
MRPSEATVYLPPVPVSKVVSTDEYVTRTNIYYHAGSARLLTVGHPYYSIPKSDNPKKIVVPKVSGLQYRVFRVRLPDPNKFGFPDTSFYNPETQRLVWACVGLEVGRGQPLGVGISGHPLLNKFDDTENSNRGPLYKTCKQAGTCPPDVIPGPGTDNRECISMDYKQTQLCLLGCKPPIGEHWGKGSPCSNNAITPGDCPPLELKNSVIQDGDMVDTGFGAMDFTALQDTKSNVPLDICNSICKYPDYLKMVAEPYGDTLFFYLRREQMFVRHFFNRSGTVGESVPNDLYIKGSGSTATLANSTYFPTPSGSMVTSDAQIFNKPYWMQRAQGHNNGICWGNQLFVTVVDTTRSTNMSVCAAIANSDTTFKSSNFKEYLRHGEEFDLQFIFQLCKITLSADIMTYIHSMNPAILEDWNFGLTTPPSGSLEDTYRFVTSQAITCQKTAPQKPKEDPFKDYVFWEVNLKEKFSADLDQFPLGRKFLLQAGY

SEQ ID NO: 20 - protein, 521 aa, Artificial Sequence
  PEPTIDE (1)..(521): 31L1DE132-136/dE-CS1
MRPSEATVYLPPVPVSKVVSTDEYVTRTNIYYHAGSARLLTVGHPYYSIPKSDNPKKIVVPKVSGLQYRVFRVRLPDPNKFGFPDTSFYNPETQRLVWACVGLEVGRGQPLGVGISGHPLLNKFDDTENSNRGPQLYKTCKQAGTCPPDVIPKVEGPGTDNRECISMDYKQTQLCLLGCKPPIGEHWGKGSPCSNNAITPGDCPPLELKNSVIQDGDMVDTGFGAMDFTALQDTKSNVPLDICNSICKYPDYLKMVAEPYGDTLFFYLRREQMFVRHFFNRSGTVGESVPNDLYIKGSGSTATLANSTYFPTPSGSMVTSDAQIFNKPYWMQRAQGHNNGICWGNQLFVTVVDTTRSTNMSVCAAIANSDTTFKSSNFKEYLRHGEEFDLQFIFQLCKITLSADIMTYIHSMNPAILEDWNFGLTTPPSGSLEDTYRFVTSQAITCQKTAPQKPKEDPFKDYVFWEVNLKEKFSADLDQFPLGRKFLLQAGYRAGPSFAAGAGSAPSASTTTPAGGSATGS

SEQ ID NO: 21 - protein, 517 aa, Artificial Sequence
  PEPTIDE (1)..(521): 31L1DE132-136/dES-CS1
MRPSEATVYLPPVPVSKVVSTDEYVTRTNIYYHAGSARLLTVGHPYYSIPKSDNPKKIVVPKVSGLQYRVFRVRLPDPNKFGFPDTSFYNPETQRLVWACVGLEVGRGQPLGVGISGHPLLNKFDDTENSNRGPLYKTCKQAGTCPPDVIPGPGTDNRECISMDYKQTQLCLLGCKPPIGEHWGKGSPCSNNAITPGDCPPLELKNSVIQDGDMVDTGFGAMDFTALQDTKSNVPLDICNSICKYPDYLKMVAEPYGDTLFFYLRREQMFVRHFFNRSGTVGESVPNDLYIKGSGSTATLANSTYFPTPSGSMVTSDAQIFNKPYWMQRAQGHNNGICWGNQLFVTVVDTTRSTNMSVCAAIANSDTTFKSSNFKEYLRHGEEFDLQFIFQLCKITLSADIMTYIHSMNPAILEDWNFGLTTPPSGSLEDTYRFVTSQAITCQKTAPQKPKEDPFKDYVFWEVNLKEKFSADLDQFPLGRKFLLQAGYRAGPSFAAGAGSAPSASTTTPAGGSATGS

SEQ ID NO: 22 - protein, 521 aa, Artificial Sequence
  PEPTIDE (1)..(521): 31L1DE132-136/dE-CS2
MRPSEATVYLPPVPVSKVVSTDEYVTRTNIYYHAGSARLLTVGHPYYSIPKSDNPKKIVVPKVSGLQYRVFRVRLPDPNKFGFPDTSFYNPETQRLVWACVGLEVGRGQPLGVGISGHPLLNKFDDTENSNRGPQLYKTCKQAGTCPPDVIPKVEGPGTDNRECISMDYKQTQLCLLGCKPPIGEHWGKGSPCSNNAITPGDCPPLELKNSVIQDGDMVDTGFGAMDFTALQDTKSNVPLDICNSICKYPDYLKMVAEPYGDTLFFYLRREQMFVRHFFNRSGTVGESVPNDLYIKGSGSTATLANSTYFPTPSGSMVTSDAQIFNKPYWMQRAQGHNNGICWGNQLFVTVVDTTRSTNMSVCAAIANSDTTFKSSNFKEYLRHGEEFDLQFIFQLCKITLSADIMTYIHSMNPAILEDWNFGLTTPPSGSLEDTYRFVTSQAITCQKTAPQKPKEDPFKDYVFWEVNLKEKFSADLDQFPLGRKFLLQAGYGAGPSFAAGAGSAPSASTTTPAGGSATGS

SEQ ID NO: 23 - protein, 517 aa, Artificial Sequence
  PEPTIDE (1)..(517): 31L1DE132-136/dES-CS2
MRPSEATVYLPPVPVSKVVSTDEYVTRTNIYYHAGSARLLTVGHPYYSIPKSDNPKKIVVPKVSGLQYRVFRVRLPDPNKFGFPDTSFYNPETQRLVWACVGLEVGRGQPLGVGISGHPLLNKFDDTENSNRGPLYKTCKQAGTCPPDVIPGPGTDNRECISMDYKQTQLCLLGCKPPIGEHWGKGSPCSNNAITPGDCPPLELKNSVIQDGDMVDTGFGAMDFTALQDTKSNVPLDICNSICKYPDYLKMVAEPYGDTLFFYLRREQMFVRHFFNRSGTVGESVPNDLYIKGSGSTATLANSTYFPTPSGSMVTSDAQIFNKPYWMQRAQGHNNGICWGNQLFVTVVDTTRSTNMSVCAAIANSDTTFKSSNFKEYLRHGEEFDLQFIFQLCKITLSADIMTYIHSMNPAILEDWNFGLTTPPSGSLEDTYRFVTSQAITCQKTAPQKPKEDPFKDYVFWEVNLKEKFSADLDQFPLGRKFLLQAGYGAGPSFAAGAGSAPSASTTTPAGGSATGS

SEQ ID NO: 24 - protein, 521 aa, Artificial Sequence
  PEPTIDE (1)..(521): 31L1DE132-136/dE-CS3
MRPSEATVYLPPVPVSKVVSTDEYVTRTNIYYHAGSARLLTVGHPYYSIPKSDNPKKIVVPKVSGLQYRVFRVRLPDPNKFGFPDTSFYNPETQRLVWACVGLEVGRGQPLGVGISGHPLLNKFDDTENSNRGPQLYKTCKQAGTCPPDVIPKVEGPGTDNRECISMDYKQTQLCLLGCKPPIGEHWGKGSPCSNNAITPGDCPPLELKNSVIQDGDMVDTGFGAMDFTALQDTKSNVPLDICNSICKYPDYLKMVAEPYGDTLFFYLRREQMFVRHFFNRSGTVGESVPNDLYIKGSGSTATLANSTYFPTPSGSMVTSDAQIFNKPYWMQRAQGHNNGICWGNQLFVTVVDTTRSTNMSVCAAIANSDTTFKSSNFKEYLRHGEEFDLQFIFQLCKITLSADIMTYIHSMNPAILEDWNFGLTTPPSGSLEDTYRFVTSQAITCQKTAPQKPKEDPFKDYVFWEVNLKEKFSADLDQFPLGRKFLLQAGYRAGPSFKAGAGSAPSASTTTPAGGSATGS

SEQ ID NO: 25 - protein, 517 aa, Artificial Sequence
  PEPTIDE (1)..(517): 31L1DE132-136/dES-CS3
MRPSEATVYLPPVPVSKVVSTDEYVTRTNIYYHAGSARLLTVGHPYYSIPKSDNPKKIVVPKVSGLQYRVFRVRLPDPNKFGFPDTSFYNPETQRLVWACVGLEVGRGQPLGVGISGHPLLNKFDDTENSNRGPLYKTCKQAGTCPPDVIPGPGTDNRECISMDYKQTQLCLLGCKPPIGEHWGKGSPCSNNAITPGDCPPLELKNSVIQDGDMVDTGFGAMDFTALQDTKSNVPLDICNSICKYPDYLKMVAEPYGDTLFFYLRREQMFVRHFFNRSGTVGESVPNDLYIKGSGSTATLANSTYFPTPSGSMVTSDAQIFNKPYWMQRAQGHNNGICWGNQLFVTVVDTTRSTNMSVCAAIANSDTTFKSSNFKEYLRHGEEFDLQFIFQLCKITLSADIMTYIHSMNPAILEDWNFGLTTPPSGSLEDTYRFVTSQAITCQKTAPQKPKEDPFKDYVFWEVNLKEKFSADLDQFPLGRKFLLQAGYRAGPSFKAGAGSAPSASTTTPAGGSATGS

SEQ ID NO: 26 - protein, 491 aa, Artificial Sequence
  PEPTIDE (1)..(491): 31L1h4428-431/dE
MRPSEATVYLPPVPVSKVVSTDEYVTRTNIYYHAGSARLLTVGHPYYSIPKSDNPKKIVVPKVSGLQYRVFRVRLPDPNKFGFPDTSFYNPETQRLVWACVGLEVGRGQPLGVGISGHPLLNKFDDTENSNRYAGGPGTDNRECISMDYKQTQLCLLGCKPPIGEHWGKGSPCSNNAITPGDCPPLELKNSVIQDGDMVDTGFGAMDFTALQDTKSNVPLDICNSICKYPDYLKMVAEPYGDTLFFYLRREQMFVRHFFNRSGTVGESVPNDLYIKGSGSTATLANSTYFPTPSGSMVTSDAQIFNKPYWMQRAQGHNNGICWGNQLFVTVVDTTRSTNMSVCAAIANSDTTFKSSNFKEYLRHGEEFDLQFIFQLCKITLSADIMTYIHSMNPAILEDWNFGLTTPPSGSLEDTYRFVTSQAITCQKLYKTCKQAGTCPPDVIPKVEGPQKPKEDPFKDYVFWEVNLKEKFSADLDQFPLGRKFLLQAGY

SEQ ID NO: 27 - protein, 487 aa, Artificial Sequence
  PEPTIDE (1)..(487): 31L1h4428-431/dES
MRPSEATVYLPPVPVSKVVSTDEYVTRTNIYYHAGSARLLTVGHPYYSIPKSDNPKKIVVPKVSGLQYRVFRVRLPDPNKFGFPDTSFYNPETQRLVWACVGLEVGRGQPLGVGISGHPLLNKFDDTENSNRYAGGPGTDNRECISMDYKQTQLCLLGCKPPIGEHWGKGSPCSNNAITPGDCPPLELKNSVIQDGDMVDTGFGAMDFTALQDTKSNVPLDICNSICKYPDYLKMVAEPYGDTLFFYLRREQMFVRHFFNRSGTVGESVPNDLYIKGSGSTATLANSTYFPTPSGSMVTSDAQIFNKPYWMQRAQGHNNGICWGNQLFVTVVDTTRSTNMSVCAAIANSDTTFKSSNFKEYLRHGEEFDLQFIFQLCKITLSADIMTYIHSMNPAILEDWNFGLTTPPSGSLEDTYRFVTSQAITCQKLYKTCKQAGTCPPDVIPPQKPKEDPFKDYVFWEVNLKEKFSADLDQFPLGRKFLLQAGY

SEQ ID NO: 28 - protein, 520 aa, Artificial Sequence
  PEPTIDE (1)..(520): 31L1h4428-431/dE-CS1
MRPSEATVYLPPVPVSKVVSTDEYVTRTNIYYHAGSARLLTVGHPYYSIPKSDNPKKIVVPKVSGLQYRVFRVRLPDPNKFGFPDTSFYNPETQRLVWACVGLEVGRGQPLGVGISGHPLLNKFDDTENSNRYAGGPGTDNRECISMDYKQTQLCLLGCKPPIGEHWGKGSPCSNNAITPGDCPPLELKNSVIQDGDMVDTGFGAMDFTALQDTKSNVPLDICNSICKYPDYLKMVAEPYGDTLFFYLRREQMFVRHFFNRSGTVGESVPNDLYIKGSGSTATLANSTYFPTPSGSMVTSDAQIFNKPYWMQRAQGHNNGICWGNQLFVTVVDTTRSTNMSVCAAIANSDTTFKSSNFKEYLRHGEEFDLQFIFQLCKITLSADIMTYIHSMNPAILEDWNFGLTTPPSGSLEDTYRFVTSQAITCQKLYKTCKQAGTCPPDVIPKVEGPQKPKEDPFKDYVFWEVNLKEKFSADLDQFPLGRKFLLQAGYRAGPSFAAGAGSAPSASTTTPAGGSATGS

SEQ ID NO: 29 - protein, 516 aa, Artificial Sequence
  PEPTIDE (1)..(516): 31L1h4428-431/dES-CS1
MRPSEATVYLPPVPVSKVVSTDEYVTRTNIYYHAGSARLLTVGHPYYSIPKSDNPKKIVVPKVSGLQYRVFRVRLPDPNKFGFPDTSFYNPETQRLVWACVGLEVGRGQPLGVGISGHPLLNKFDDTENSNRYAGGPGTDNRECISMDYKQTQLCLLGCKPPIGEHWGKGSPCSNNAITPGDCPPLELKNSVIQDGDMVDTGFGAMDFTALQDTKSNVPLDICNSICKYPDYLKMVAEPYGDTLFFYLRREQMFVRHFFNRSGTVGESVPNDLYIKGSGSTATLANSTYFPTPSGSMVTSDAQIFNKPYWMQRAQGHNNGICWGNQLFVTVVDTTRSTNMSVCAAIANSDTTFKSSNFKEYLRHGEEFDLQFIFQLCKITLSADIMTYIHSMNPAILEDWNFGLTTPPSGSLEDTYRFVTSQAITCQKLYKTCKQAGTCPPDVIPPQKPKEDPFKDYVFWEVNLKEKFSADLDQFPLGRKFLLQAGYRAGPSFAAGAGSAPSASTTTPAGGSATGS

SEQ ID NO: 30 - protein, 520 aa, Artificial Sequence
  PEPTIDE (1)..(520): 31L1h4428-431/dE-CS2
MRPSEATVYLPPVPVSKVVSTDEYVTRTNIYYHAGSARLLTVGHPYYSIPKSDNPKKIVVPKVSGLQYRVFRVRLPDPNKFGFPDTSFYNPETQRLVWACVGLEVGRGQPLGVGISGHPLLNKFDDTENSNRYAGGPGTDNRECISMDYKQTQLCLLGCKPPIGEHWGKGSPCSNNAITPGDCPPLELKNSVIQDGDMVDTGFGAMDFTALQDTKSNVPLDICNSICKYPDYLKMVAEPYGDTLFFYLRREQMFVRHFFNRSGTVGESVPNDLYIKGSGSTATLANSTYFPTPSGSMVTSDAQIFNKPYWMQRAQGHNNGICWGNQLFVTVVDTTRSTNMSVCAAIANSDTTFKSSNFKEYLRHGEEFDLQFIFQLCKITLSADIMTYIHSMNPAILEDWNFGLTTPPSGSLEDTYRFVTSQAITCQKLYKTCKQAGTCPPDVIPKVEGPQKPKEDPFKDYVFWEVNLKEKFSADLDQFPLGRKFLLQAGYGAGPSFAAGAGSAPSASTTTPAGGSATGS

SEQ ID NO: 31 - protein, 516 aa, Artificial Sequence
  PEPTIDE (1)..(516): 31L1h4428-431/dES-CS2
MRPSEATVYLPPVPVSKVVSTDEYVTRTNIYYHAGSARLLTVGHPYYSIPKSDNPKKIVVPKVSGLQYRVFRVRLPDPNKFGFPDTSFYNPETQRLVWACVGLEVGRGQPLGVGISGHPLLNKFDDTENSNRYAGGPGTDNRECISMDYKQTQLCLLGCKPPIGEHWGKGSPCSNNAITPGDCPPLELKNSVIQDGDMVDTGFGAMDFTALQDTKSNVPLDICNSICKYPDYLKMVAEPYGDTLFFYLRREQMFVRHFFNRSGTVGESVPNDLYIKGSGSTATLANSTYFPTPSGSMVTSDAQIFNKPYWMQRAQGHNNGICWGNQLFVTVVDTTRSTNMSVCAAIANSDTTFKSSNFKEYLRHGEEFDLQFIFQLCKITLSADIMTYIHSMNPAILEDWNFGLTTPPSGSLEDTYRFVTSQAITCQKLYKTCKQAGTCPPDVIPPQKPKEDPFKDYVFWEVNLKEKFSADLDQFPLGRKFLLQAGYGAGPSFAAGAGSAPSASTTTPAGGSATGS

SEQ ID NO: 32 - protein, 520 aa, Artificial Sequence
  PEPTIDE (1)..(520): 31L1h4428-431/dE-CS3
MRPSEATVYLPPVPVSKVVSTDEYVTRTNIYYHAGSARLLTVGHPYYSIPKSDNPKKIVVPKVSGLQYRVFRVRLPDPNKFGFPDTSFYNPETQRLVWACVGLEVGRGQPLGVGISGHPLLNKFDDTENSNRYAGGPGTDNRECISMDYKQTQLCLLGCKPPIGEHWGKGSPCSNNAITPGDCPPLELKNSVIQDGDMVDTGFGAMDFTALQDTKSNVPLDICNSICKYPDYLKMVAEPYGDTLFFYLRREQMFVRHFFNRSGTVGESVPNDLYIKGSGSTATLANSTYFPTPSGSMVTSDAQIFNKPYWMQRAQGHNNGICWGNQLFVTVVDTTRSTNMSVCAAIANSDTTFKSSNFKEYLRHGEEFDLQFIFQLCKITLSADIMTYIHSMNPAILEDWNFGLTTPPSGSLEDTYRFVTSQAITCQKLYKTCKQAGTCPPDVIPKVEGPQKPKEDPFKDYVFWEVNLKEKFSADLDQFPLGRKFLLQAGYRAGPSFKAGAGSAPSASTTTPAGGSATGS

SEQ ID NO: 33 - protein, 516 aa, Artificial Sequence
  PEPTIDE (1)..(516): 31L1h4428-431/dES-CS3
MRPSEATVYLPPVPVSKVVSTDEYVTRTNIYYHAGSARLLTVGHPYYSIPKSDNPKKIVVPKVSGLQYRVFRVRLPDPNKFGFPDTSFYNPETQRLVWACVGLEVGRGQPLGVGISGHPLLNKFDDTENSNRYAGGPGTDNRECISMDYKQTQLCLLGCKPPIGEHWGKGSPCSNNAITPGDCPPLELKNSVIQDGDMVDTGFGAMDFTALQDTKSNVPLDICNSICKYPDYLKMVAEPYGDTLFFYLRREQMFVRHFFNRSGTVGESVPNDLYIKGSGSTATLANSTYFPTPSGSMVTSDAQIFNKPYWMQRAQGHNNGICWGNQLFVTVVDTTRSTNMSVCAAIANSDTTFKSSNFKEYLRHGEEFDLQFIFQLCKITLSADIMTYIHSMNPAILEDWNFGLTTPPSGSLEDTYRFVTSQAITCQKLYKTCKQAGTCPPDVIPPQKPKEDPFKDYVFWEVNLKEKFSADLDQFPLGRKFLLQAGYRAGPSFKAGAGSAPSASTTTPAGGSATGS

SEQ ID NO: 34 - DNA, 1429 bp, Artificial Sequence
  gene (1)..(1429): 31L1 delta C29 nt
atgagcctgtggagaccatcagaggctacagtatatctgccacctgttcctgtaagcaaagtggtttcaaccgatgagtacgtaacacgtaccaacatctactatcacgctggatctgcgcgcctcctgactgtcggtcacccatactactctattcccaagtcagacaatcccaagaaaatcgtggtacccaaagtgagcggactccagtatcgtgttttcagagtccgcttgccagatcccaacaagtttggcttcccagacacaagcttctacaatcctgaaacccaacgcctggtatgggcatgcgtgggactcgaggttggccgtggtcagcctctgggagtgggcatctcaggccacccattgctcaacaaattcgatgacaccgagaattccaacagatacgcgggtggaccaggtacagataaccgcgaatgcatcagcatggactacaagcagacccaactgtgcctcttgggctgcaagccaccaattggagagcactggggcaaaggctcaccttgctccaacaacgctatcacacctggagactgcccacccttggaactcaagaattctgtcattcaggatggtgacatggtggacactggctttggtgcaatggatttcaccgctcttcaagacaccaagtcaaacgtacctctggatatctgcaatagcatttgcaagtatccagactacctcaagatggttgctgagccttacggtgatacactgttcttctacctgagacgtgagcagatgtttgtgagacacttcttcaaccgttccggcactgtcggagagtcagttcctacagacctctacatcaagggttctggcagcacagcaactctggcgaactcaacctactttcctactccttccggatctatggtcacgagcgatgctcagatcttcaacaagccctactggatgcaacgtgcccagggacacaacaatggcatttgctggggcaatcagctcttcgtcactgttgtggacactactcgctccactaacatgtctgtctgcgctgccattgccaactccgataccactttcaaaagctctaactttaaggaatatctgcgtcacggtgaggagttcgacttgcagttcatcttccaactctgcaagatcaccctgtccgctgatatcatgacctacattcacagcatgaatccagctatcctggaagactggaacttcggtctgaccactccaccctctggtagcctggaggatacctacaggtttgttacatctcaagcaatcacttgccagaagactgccccacagaagcctaaagaggaccccttcaaagattacgtcttctgggaggtgaatctgaaggagaagttctctgctgatttggatcagtttccactgggtcgtaagttcctgctccaagctggatactaag

SEQ ID NO: 35 - DNA, 1429 bp, Artificial Sequence
  gene (1)..(1428): T274N delta C29 nt
atgagcctgtggagaccatcagaggctacagtatatctgccacctgttcctgtaagcaaagtggtttcaaccgatgagtacgtaacacgtaccaacatctactatcacgctggatctgcgcgcctcctgactgtcggtcacccatactactctattcccaagtcagacaatcccaagaaaatcgtggtacccaaagtgagcggactccagtatcgtgttttcagagtccgcttgccagatcccaacaagtttggcttcccagacacaagcttctacaatcctgaaacccaacgcctggtatgggcatgcgtgggactcgaggttggccgtggtcagcctctgggagtgggcatctcaggccacccattgctcaacaaattcgatgacaccgagaattccaacagatacgcgggtggaccaggtacagataaccgcgaatgcatcagcatggactacaagcagacccaactgtgcctcttgggctgcaagccaccaattggagagcactggggcaaaggctcaccttgctccaacaacgctatcacacctggagactgcccacccttggaactcaagaattctgtcattcaggatggtgacatggtggacactggctttggtgcaatggatttcaccgctcttcaagacaccaagtcaaacgtacctctggatatctgcaatagcatttgcaagtatccagactacctcaagatggttgctgagccttacggtgatacactgttcttctacctgagacgtgagcagatgtttgtgagacacttcttcaaccgttccggcactgtcggagagtcagttcctaacgacctctacatcaagggttctggcagcacagcaactctggcgaactcaacctactttcctactccttccggatctatggtcacgagcgatgctcagatcttcaacaagccctactggatgcaacgtgcccagggacacaacaatggcatttgctggggcaatcagctcttcgtcactgttgtggacactactcgctccactaacatgtctgtctgcgctgccattgccaactccgataccactttcaaaagctctaactttaaggaatatctgcgtcacggtgaggagttcgacttgcagttcatcttccaactctgcaagatcaccctgtccgctgatatcatgacctacattcacagcatgaatccagctatcctggaagactggaacttcggtctgaccactccaccctctggtagcctggaggatacctacaggtttgttacatctcaagcaatcacttgccagaagactgccccacagaagcctaaagaggaccccttcaaagattacgtcttctgggaggtgaatctgaaggagaagttctctgctgatttggatcagtttccactgggtcgtaagttcctgctccaagctggatactaag

SEQ ID NO: 36 - DNA, 1420 bp, Artificial Sequence
  gene (1)..(1420): T274N delta N4C29
atgagaccatcagaggctacagtatatctgccacctgttcctgtaagcaaagtggtttcaaccgatgagtacgtaacacgtaccaacatctactatcacgctggatctgcgcgcctcctgactgtcggtcacccatactactctattcccaagtcagacaatcccaagaaaatcgtggtacccaaagtgagcggactccagtatcgtgttttcagagtccgcttgccagatcccaacaagtttggcttcccagacacaagcttctacaatcctgaaacccaacgcctggtatgggcatgcgtgggactcgaggttggccgtggtcagcctctgggagtgggcatctcaggccacccattgctcaacaaattcgatgacaccgagaattccaacagatacgcgggtggaccaggtacagataaccgcgaatgcatcagcatggactacaagcagacccaactgtgcctcttgggctgcaagccaccaattggagagcactggggcaaaggctcaccttgctccaacaacgctatcacacctggagactgcccacccttggaactcaagaattctgtcattcaggatggtgacatggtggacactggctttggtgcaatggatttcaccgctcttcaagacaccaagtcaaacgtacctctggatatctgcaatagcatttgcaagtatccagactacctcaagatggttgctgagccttacggtgatacactgttcttctacctgagacgtgagcagatgtttgtgagacacttcttcaaccgttccggcactgtcggagagtcagttcctaacgacctctacatcaagggttctggcagcacagcaactctggcgaactcaacctactttcctactccttccggatctatggtcacgagcgatgctcagatcttcaacaagccctactggatgcaacgtgcccagggacacaacaatggcatttgctggggcaatcagctcttcgtcactgttgtggacactactcgctccactaacatgtctgtctgcgctgccattgccaactccgataccactttcaaaagctctaactttaaggaatatctgcgtcacggtgaggagttcgacttgcagttcatcttccaactctgcaagatcaccctgtccgctgatatcatgacctacattcacagcatgaatccagctatcctggaagactggaacttcggtctgaccactccaccctctggtagcctggaggatacctacaggtttgttacatctcaagcaatcacttgccagaagactgccccacagaagcctaaagaggaccccttcaaagattacgtcttctgggaggtgaatctgaaggagaagttctctgctgatttggatcagtttccactgggtcgtaagttcctgctccaagctggatactaag

SEQ ID NO: 37 - DNA, 1480 bp, Artificial Sequence
  gene (1)..(1480): 31L1DE132-136/dE nt
atgagaccatcagaggctacagtatatctgccacctgttcctgtaagcaaagtggtttcaaccgatgagtacgtaacacgtaccaacatctactatcacgctggatctgcgcgcctcctgactgtcggtcacccatactactctattcccaagtcagacaatcccaagaaaatcgtggtacccaaagtgagcggactccagtatcgtgttttcagagtccgcttgccagatcccaacaagtttggcttcccagacacaagcttctacaatcctgaaacccaacgcctggtatgggcatgcgtgggactcgaggttggccgtggtcagcctctgggagtgggcatctcaggccacccattgctcaacaaattcgatgacaccgagaattccaacagaggtcctcagctgtacaagacctgcaagcaggctggtacctgccctcctgacgtgatccctaaggtggagggaccaggtacagataaccgcgaatgcatcagcatggactacaagcagacccaactgtgcctcttgggctgcaagccaccaattggagagcactggggcaaaggctcaccttgctccaacaacgctatcacacctggagactgcccacccttggaactcaagaattctgtcattcaggatggtgacatggtggacactggctttggtgcaatggatttcaccgctcttcaagacaccaagtcaaacgtacctctggatatctgcaatagcatttgcaagtatccagactacctcaagatggttgctgagccttacggtgatacactgttcttctacctgagacgtgagcagatgtttgtgagacacttcttcaaccgttccggcactgtcggagagtcagttcctaacgacctctacatcaagggttctggcagcacagcaactctggcgaactcaacctactttcctactccttccggatctatggtcacgagcgatgctcagatcttcaacaagccctactggatgcaacgtgcccagggacacaacaatggcatttgctggggcaatcagctcttcgtcactgttgtggacactactcgctccactaacatgtctgtctgcgctgccattgccaactccgataccactttcaaaagctctaactttaaggaatatctgcgtcacggtgaggagttcgacttgcagttcatcttccaactctgcaagatcaccctgtccgctgatatcatgacctacattcacagcatgaatccagctatcctggaagactggaacttcggtctgaccactccaccctctggtagcctggaggatacctacaggtttgttacatctcaagcaatcacttgccagaagactgccccacagaagcctaaagaggaccccttcaaagattacgtcttctgggaggtgaatctgaaggagaagttctctgctgatttggatcagtttccactgggtcgtaagttcctgctccaagctggatactaag

SEQ ID NO: 38 - DNA, 1468 bp, Artificial Sequence
  gene (1)..(1468): 31L1DE132-136/dES nt
atgagaccatcagaggctacagtatatctgccacctgttcctgtaagcaaagtggtttcaaccgatgagtacgtaacacgtaccaacatctactatcacgctggatctgcgcgcctcctgactgtcggtcacccatactactctattcccaagtcagacaatcccaagaaaatcgtggtacccaaagtgagcggactccagtatcgtgttttcagagtccgcttgccagatcccaacaagtttggcttcccagacacaagcttctacaatcctgaaacccaacgcctggtatgggcatgcgtgggactcgaggttggccgtggtcagcctctgggagtgggcatctcaggccacccattgctcaacaaattcgatgacaccgagaattccaacagaggtcctctgtacaagacctgcaagcaggctggtacctgccctcctgacgtgatccctggaccaggtacagataaccgcgaatgcatcagcatggactacaagcagacccaactgtgcctcttgggctgcaagccaccaattggagagcactggggcaaaggctcaccttgctccaacaacgctatcacacctggagactgcccacccttggaactcaagaattctgtcattcaggatggtgacatggtggacactggctttggtgcaatggatttcaccgctcttcaagacaccaagtcaaacgtacctctggatatctgcaatagcatttgcaagtatccagactacctcaagatggttgctgagccttacggtgatacactgttcttctacctgagacgtgagcagatgtttgtgagacacttcttcaaccgttccggcactgtcggagagtcagttcctaacgacctctacatcaagggttctggcagcacagcaactctggcgaactcaacctactttcctactccttccggatctatggtcacgagcgatgctcagatcttcaacaagccctactggatgcaacgtgcccagggacacaacaatggcatttgctggggcaatcagctcttcgtcactgttgtggacactactcgctccactaacatgtctgtctgcgctgccattgccaactccgataccactttcaaaagctctaactttaaggaatatctgcgtcacggtgaggagttcgacttgcagttcatcttccaactctgcaagatcaccctgtccgctgatatcatgacctacattcacagcatgaatccagctatcctggaagactggaacttcggtctgaccactccaccctctggtagcctggaggatacctacaggtttgttacatctcaagcaatcacttgccagaagactgccccacagaagcctaaagaggaccccttcaaagattacgtcttctgggaggtgaatctgaaggagaagttctctgctgatttggatcagtttccactgggtcgtaagttcctgctccaagctggatactaag

SEQ ID NO: 39 - DNA, 1567 bp, Artificial Sequence
  gene (1)..(1567): 31L1DE132-136/dE-CS1 nt
atgagaccatcagaggctacagtatatctgccacctgttcctgtaagcaaagtggtttcaaccgatgagtacgtaacacgtaccaacatctactatcacgctggatctgcgcgcctcctgactgtcggtcacccatactactctattcccaagtcagacaatcccaagaaaatcgtggtacccaaagtgagcggactccagtatcgtgttttcagagtccgcttgccagatcccaacaagtttggcttcccagacacaagcttctacaatcctgaaacccaacgcctggtatgggcatgcgtgggactcgaggttggccgtggtcagcctctgggagtgggcatctcaggccacccattgctcaacaaattcgatgacaccgagaattccaacagaggtcctcagctgtacaagacctgcaagcaggctggtacctgccctcctgacgtgatccctaaggtggagggaccaggtacagataaccgcgaatgcatcagcatggactacaagcagacccaactgtgcctcttgggctgcaagccaccaattggagagcactggggcaaaggctcaccttgctccaacaacgctatcacacctggagactgcccacccttggaactcaagaattctgtcattcaggatggtgacatggtggacactggctttggtgcaatggatttcaccgctcttcaagacaccaagtcaaacgtacctctggatatctgcaatagcatttgcaagtatccagactacctcaagatggttgctgagccttacggtgatacactgttcttctacctgagacgtgagcagatgtttgtgagacacttcttcaaccgttccggcactgtcggagagtcagttcctaacgacctctacatcaagggttctggcagcacagcaactctggcgaactcaacctactttcctactccttccggatctatggtcacgagcgatgctcagatcttcaacaagccctactggatgcaacgtgcccagggacacaacaatggcatttgctggggcaatcagctcttcgtcactgttgtggacactactcgctccactaacatgtctgtctgcgctgccattgccaactccgataccactttcaaaagctctaactttaaggaatatctgcgtcacggtgaggagttcgacttgcagttcatcttccaactctgcaagatcaccctgtccgctgatatcatgacctacattcacagcatgaatccagctatcctggaagactggaacttcggtctgaccactccaccctctggtagcctggaggatacctacaggtttgttacatctcaagcaatcacttgccagaagactgccccacagaagcctaaagaggaccccttcaaagattacgtcttctgggaggtgaatctgaaggagaagttctctgctgatttggatcagtttccactgggtcgtaagttcctgctccaagctggataccgtgctggtccttcgtttgccgctggcgcgggttcggctcctagcgcctcgactaccacgccggctggcggttcggccacgggcagctaag

SEQ ID NO: 40 - DNA, 1555 bp, Artificial Sequence
  gene (1)..(1555): 31L1DE132-136/dES-CS1 nt
atgagaccatcagaggctacagtatatctgccacctgttcctgtaagcaaagtggtttcaaccgatgagtacgtaacacgtaccaacatctactatcacgctggatctgcgcgcctcctgactgtcggtcacccatactactctattcccaagtcagacaatcccaagaaaatcgtggtacccaaagtgagcggactccagtatcgtgttttcagagtccgcttgccagatcccaacaagtttggcttcccagacacaagcttctacaatcctgaaacccaacgcctggtatgggcatgcgtgggactcgaggttggccgtggtcagcctctgggagtgggcatctcaggccacccattgctcaacaaattcgatgacaccgagaattccaacagaggtcctctgtacaagacctgcaagcaggctggtacctgccctcctgacgtgatccctggaccaggtacagataaccgcgaatgcatcagcatggactacaagcagacccaactgtgcctcttgggctgcaagccaccaattggagagcactggggcaaaggctcaccttgctccaacaacgctatcacacctggagactgcccacccttggaactcaagaattctgtcattcaggatggtgacatggtggacactggctttggtgcaatggatttcaccgctcttcaagacaccaagtcaaacgtacctctggatatctgcaatagcatttgcaagtatccagactacctcaagatggttgctgagccttacggtgatacactgttcttctacctgagacgtgagcagatgtttgtgagacacttcttcaaccgttccggcactgtcggagagtcagttcctaacgacctctacatcaagggttctggcagcacagcaactctggcgaactcaacctactttcctactccttccggatctatggtcacgagcgatgctcagatcttcaacaagccctactggatgcaacgtgcccagggacacaacaatggcatttgctggggcaatcagctcttcgtcactgttgtggacactactcgctccactaacatgtctgtctgcgctgccattgccaactccgataccactttcaaaagctctaactttaaggaatatctgcgtcacggtgaggagttcgacttgcagttcatcttccaactctgcaagatcaccctgtccgctgatatcatgacctacattcacagcatgaatccagctatcctggaagactggaacttcggtctgaccactccaccctctggtagcctggaggatacctacaggtttgttacatctcaagcaatcacttgccagaagactgccccacagaagcctaaagaggaccccttcaaagattacgtcttctgggaggtgaatctgaaggagaagttctctgctgatttggatcagtttccactgggtcgtaagttcctgctccaagctggataccgtgctggtccttcgtttgccgctggcgcgggttcggctcctagcgcctcgactaccacgccggctggcggttcggccacgggcagctaag

SEQ ID NO: 41 - DNA, 1567 bp, Artificial Sequence
  gene (1)..(1567): 31L1DE132-136/dE-CS2 nt
atgagaccatcagaggctacagtatatctgccacctgttcctgtaagcaaagtggtttcaaccgatgagtacgtaacacgtaccaacatctactatcacgctggatctgcgcgcctcctgactgtcggtcacccatactactctattcccaagtcagacaatcccaagaaaatcgtggtacccaaagtgagcggactccagtatcgtgttttcagagtccgcttgccagatcccaacaagtttggcttcccagacacaagcttctacaatcctgaaacccaacgcctggtatgggcatgcgtgggactcgaggttggccgtggtcagcctctgggagtgggcatctcaggccacccattgctcaacaaattcgatgacaccgagaattccaacagaggtcctcagctgtacaagacctgcaagcaggctggtacctgccctcctgacgtgatccctaaggtggagggaccaggtacagataaccgcgaatgcatcagcatggactacaagcagacccaactgtgcctcttgggctgcaagccaccaattggagagcactggggcaaaggctcaccttgctccaacaacgctatcacacctggagactgcccacccttggaactcaagaattctgtcattcaggatggtgacatggtggacactggctttggtgcaatggatttcaccgctcttcaagacaccaagtcaaacgtacctctggatatctgcaatagcatttgcaagtatccagactacctcaagatggttgctgagccttacggtgatacactgttcttctacctgagacgtgagcagatgtttgtgagacacttcttcaaccgttccggcactgtcggagagtcagttcctaacgacctctacatcaagggttctggcagcacagcaactctggcgaactcaacctactttcctactccttccggatctatggtcacgagcgatgctcagatcttcaacaagccctactggatgcaacgtgcccagggacacaacaatggcatttgctggggcaatcagctcttcgtcactgttgtggacactactcgctccactaacatgtctgtctgcgctgccattgccaactccgataccactttcaaaagctctaactttaaggaatatctgcgtcacggtgaggagttcgacttgcagttcatcttccaactctgcaagatcaccctgtccgctgatatcatgacctacattcacagcatgaatccagctatcctggaagactggaacttcggtctgaccactccaccctctggtagcctggaggatacctacaggtttgttacatctcaagcaatcacttgccagaagactgccccacagaagcctaaagaggaccccttcaaagattacgtcttctgggaggtgaatctgaaggagaagttctctgctgatttggatcagtttccactgggtcgtaagttcctgctccaagctggatacggcgctggtccttcgtttgccgctggcgcgggttcggctcctagcgcctcgactaccacgccggctggcggttcggccacgggcagctaag

SEQ ID NO: 42 - DNA, 1555 bp, Artificial Sequence
  gene (1)..(1555): 31L1DE132-136/dES-CS2 nt
atgagaccatcagaggctacagtatatctgccacctgttcctgtaagcaaagtggtttcaaccgatgagtacgtaacacgtaccaacatctactatcacgctggatctgcgcgcctcctgactgtcggtcacccatactactctattcccaagtcagacaatcccaagaaaatcgtggtacccaaagtgagcggactccagtatcgtgttttcagagtccgcttgccagatcccaacaagtttggcttcccagacacaagcttctacaatcctgaaacccaacgcctggtatgggcatgcgtgggactcgaggttggccgtggtcagcctctgggagtgggcatctcaggccacccattgctcaacaaattcgatgacaccgagaattccaacagaggtcctctgtacaagacctgcaagcaggctggtacctgccctcctgacgtgatccctggaccaggtacagataaccgcgaatgcatcagcatggactacaagcagacccaactgtgcctcttgggctgcaagccaccaattggagagcactggggcaaaggctcaccttgctccaacaacgctatcacacctggagactgcccacccttggaactcaagaattctgtcattcaggatggtgacatggtggacactggctttggtgcaatggatttcaccgctcttcaagacaccaagtcaaacgtacctctggatatctgcaatagcatttgcaagtatccagactacctcaagatggttgctgagccttacggtgatacactgttcttctacctgagacgtgagcagatgtttgtgagacacttcttcaaccgttccggcactgtcggagagtcagttcctaacgacctctacatcaagggttctggcagcacagcaactctggcgaactcaacctactttcctactccttccggatctatggtcacgagcgatgctcagatcttcaacaagccctactggatgcaacgtgcccagggacacaacaatggcatttgctggggcaatcagctcttcgtcactgttgtggacactactcgctccactaacatgtctgtctgcgctgccattgccaactccgataccactttcaaaagctctaactttaaggaatatctgcgtcacggtgaggagttcgacttgcagttcatcttccaactctgcaagatcaccctgtccgctgatatcatgacctacattcacagcatgaatccagctatcctggaagactggaacttcggtctgaccactccaccctctggtagcctggaggatacctacaggtttgttacatctcaagcaatcacttgccagaagactgccccacagaagcctaaagaggaccccttcaaagattacgtcttctgggaggtgaatctgaaggagaagttctctgctgatttggatcagtttccactgggtcgtaagttcctgctccaagctggatacggcgctggtccttcgtttgccgctggcgcgggttcggctcctagcgcctcgactaccacgccggctggcggttcggccacgggcagctaag

SEQ ID NO: 43 - DNA, 1567 bp, Artificial Sequence
  gene (1)..(1567): 31L1DE132-136/dE-CS3 nt
atgagaccatcagaggctacagtatatctgccacctgttcctgtaagcaaagtggtttcaaccgatgagtacgtaacacgtaccaacatctactatcacgctggatctgcgcgcctcctgactgtcggtcacccatactactctattcccaagtcagacaatcccaagaaaatcgtggtacccaaagtgagcggactccagtatcgtgttttcagagtccgcttgccagatcccaacaagtttggcttcccagacacaagcttctacaatcctgaaacccaacgcctggtatgggcatgcgtgggactcgaggttggccgtggtcagcctctgggagtgggcatctcaggccacccattgctcaacaaattcgatgacaccgagaattccaacagaggtcctcagctgtacaagacctgcaagcaggctggtacctgccctcctgacgtgatccctaaggtggagggaccaggtacagataaccgcgaatgcatcagcatggactacaagcagacccaactgtgcctcttgggctgcaagccaccaattggagagcactggggcaaaggctcaccttgctccaacaacgctatcacacctggagactgcccacccttggaactcaagaattctgtcattcaggatggtgacatggtggacactggctttggtgcaatggatttcaccgctcttcaagacaccaagtcaaacgtacctctggatatctgcaatagcatttgcaagtatccagactacctcaagatggttgctgagccttacggtgatacactgttcttctacctgagacgtgagcagatgtttgtgagacacttcttcaaccgttccggcactgtcggagagtcagttcctaacgacctctacatcaagggttctggcagcacagcaactctggcgaactcaacctactttcctactccttccggatctatggtcacgagcgatgctcagatcttcaacaagccctactggatgcaacgtgcccagggacacaacaatggcatttgctggggcaatcagctcttcgtcactgttgtggacactactcgctccactaacatgtctgtctgcgctgccattgccaactccgataccactttcaaaagctctaactttaaggaatatctgcgtcacggtgaggagttcgacttgcagttcatcttccaactctgcaagatcaccctgtccgctgatatcatgacctacattcacagcatgaatccagctatcctggaagactggaacttcggtctgaccactccaccctctggtagcctggaggatacctacaggtttgttacatctcaagcaatcacttgccagaagactgccccacagaagcctaaagaggaccccttcaaagattacgtcttctgggaggtgaatctgaaggagaagttctctgctgatttggatcagtttccactgggtcgtaagttcctgctccaagctggataccgtgctggtccttcgtttaaagctggcgcgggttcggctcctagcgcctcgactaccacgccggctggcggttcggccacgggcagctaag

SEQ ID NO: 44 - DNA, 1555 bp, Artificial Sequence
  gene (1)..(1555): 31L1DE132-136/dES-CS3 nt
atgagaccatcagaggctacagtatatctgccacctgttcctgtaagcaaagtggtttcaaccgatgagtacgtaacacgtaccaacatctactatcacgctggatctgcgcgcctcctgactgtcggtcacccatactactctattcccaagtcagacaatcccaagaaaatcgtggtacccaaagtgagcggactccagtatcgtgttttcagagtccgcttgccagatcccaacaagtttggcttcccagacacaagcttctacaatcctgaaacccaacgcctggtatgggcatgcgtgggactcgaggttggccgtggtcagcctctgggagtgggcatctcaggccacccattgctcaacaaattcgatgacaccgagaattccaacagaggtcctctgtacaagacctgcaagcaggctggtacctgccctcctgacgtgatccctggaccaggtacagataaccgcgaatgcatcagcatggactacaagcagacccaactgtgcctcttgggctgcaagccaccaattggagagcactggggcaaaggctcaccttgctccaacaacgctatcacacctggagactgcccacccttggaactcaagaattctgtcattcaggatggtgacatggtggacactggctttggtgcaatggatttcaccgctcttcaagacaccaagtcaaacgtacctctggatatctgcaatagcatttgcaagtatccagactacctcaagatggttgctgagccttacggtgatacactgttcttctacctgagacgtgagcagatgtttgtgagacacttcttcaaccgttccggcactgtcggagagtcagttcctaacgacctctacatcaagggttctggcagcacagcaactctggcgaactcaacctactttcctactccttccggatctatggtcacgagcgatgctcagatcttcaacaagccctactggatgcaacgtgcccagggacacaacaatggcatttgctggggcaatcagctcttcgtcactgttgtggacactactcgctccactaacatgtctgtctgcgctgccattgccaactccgataccactttcaaaagctctaactttaaggaatatctgcgtcacggtgaggagttcgacttgcagttcatcttccaactctgcaagatcaccctgtccgctgatatcatgacctacattcacagcatgaatccagctatcctggaagactggaacttcggtctgaccactccaccctctggtagcctggaggatacctacaggtttgttacatctcaagcaatcacttgccagaagactgccccacagaagcctaaagaggaccccttcaaagattacgtcttctgggaggtgaatctgaaggagaagttctctgctgatttggatcagtttccactgggtcgtaagttcctgctccaagctggataccgtgctggtccttcgtttaaagctggcgcgggttcggctcctagcgcctcgactaccacgccggctggcggttcggccacgggcagctaag

SEQ ID NO: 45 - DNA, 1477 bp, Artificial Sequence
  gene (1)..(1477): 31L1h4428-431/dE nt
atgagaccatcagaggctacagtatatctgccacctgttcctgtaagcaaagtggtttcaaccgatgagtacgtaacacgtaccaacatctactatcacgctggatctgcgcgcctcctgactgtcggtcacccatactactctattcccaagtcagacaatcccaagaaaatcgtggtacccaaagtgagcggactccagtatcgtgttttcagagtccgcttgccagatcccaacaagtttggcttcccagacacaagcttctacaatcctgaaacccaacgcctggtatgggcatgcgtgggactcgaggttggccgtggtcagcctctgggagtgggcatctcaggccacccattgctcaacaaattcgatgacaccgagaattccaacagatacgcgggtggaccaggtacagataaccgcgaatgcatcagcatggactacaagcagacccaactgtgcctcttgggctgcaagccaccaattggagagcactggggcaaaggctcaccttgctccaacaacgctatcacacctggagactgcccacccttggaactcaagaattctgtcattcaggatggtgacatggtggacactggctttggtgcaatggatttcaccgctcttcaagacaccaagtcaaacgtacctctggatatctgcaatagcatttgcaagtatccagactacctcaagatggttgctgagccttacggtgatacactgttcttctacctgagacgtgagcagatgtttgtgagacacttcttcaaccgttccggcactgtcggagagtcagttcctaacgacctctacatcaagggttctggcagcacagcaactctggcgaactcaacctactttcctactccttccggatctatggtcacgagcgatgctcagatcttcaacaagccctactggatgcaacgtgcccagggacacaacaatggcatttgctggggcaatcagctcttcgtcactgttgtggacactactcgctccactaacatgtctgtctgcgctgccattgccaactccgataccactttcaaaagctctaactttaaggaatatctgcgtcacggtgaggagttcgacttgcagttcatcttccaactctgcaagatcaccctgtccgctgatatcatgacctacattcacagcatgaatccagctatcctggaagactggaacttcggtctgaccactccaccctctggtagcctggaggatacctacaggtttgttacatctcaagcaatcacttgccagaagctgtacaagacctgcaagcaggctggtacctgccctcctgacgtgatccctaaggtggagggtccacagaagcctaaagaggaccccttcaaagattacgtcttctgggaggtgaatctgaaggagaagttctctgctgatttggatcagtttccactgggtcgtaagttcctgctccaagctggatactaag

SEQ ID NO: 46 - DNA, 1465 bp, Artificial Sequence
  gene (1)..(1465): 31L1h4428-431/dES nt
atgagaccatcagaggctacagtatatctgccacctgttcctgtaagcaaagtggtttcaaccgatgagtacgtaacacgtaccaacatctactatcacgctggatctgcgcgcctcctgactgtcggtcacccatactactctattcccaagtcagacaatcccaagaaaatcgtggtacccaaagtgagcggactccagtatcgtgttttcagagtccgcttgccagatcccaacaagtttggcttcccagacacaagcttctacaatcctgaaacccaacgcctggtatgggcatgcgtgggactcgaggttggccgtggtcagcctctgggagtgggcatctcaggccacccattgctcaacaaattcgatgacaccgagaattccaacagatacgcgggtggaccaggtacagataaccgcgaatgcatcagcatggactacaagcagacccaactgtgcctcttgggctgcaagccaccaattggagagcactggggcaaaggctcaccttgctccaacaacgctatcacacctggagactgcccacccttggaactcaagaattctgtcattcaggatggtgacatggtggacactggctttggtgcaatggatttcaccgctcttcaagacaccaagtcaaacgtacctctggatatctgcaatagcatttgcaagtatccagactacctcaagatggttgctgagccttacggtgatacactgttcttctacctgagacgtgagcagatgtttgtgagacacttcttcaaccgttccggcactgtcggagagtcagttcctaacgacctctacatcaagggttctggcagcacagcaactctggcgaactcaacctactttcctactccttccggatctatggtcacgagcgatgctcagatcttcaacaagccctactggatgcaacgtgcccagggacacaacaatggcatttgctggggcaatcagctcttcgtcactgttgtggacactactcgctccactaacatgtctgtctgcgctgccattgccaactccgataccactttcaaaagctctaactttaaggaatatctgcgtcacggtgaggagttcgacttgcagttcatcttccaactctgcaagatcaccctgtccgctgatatcatgacctacattcacagcatgaatccagctatcctggaagactggaacttcggtctgaccactccaccctctggtagcctggaggatacctacaggtttgttacatctcaagcaatcacttgccagaagctgtacaagacctgcaagcaggctggtacctgccctcctgacgtgatccctccacagaagcctaaagaggaccccttcaaagattacgtcttctgggaggtgaatctgaaggagaagttctctgctgatttggatcagtttccactgggtcgtaagttcctgctccaagctggatactaag

SEQ ID NO: 47 - DNA, 1564 bp, Artificial Sequence
  gene (1)..(1564): 31L1h4428-431/dE-CS1 nt
atgagaccatcagaggctacagtatatctgccacctgttcctgtaagcaaagtggtttcaaccgatgagtacgtaacacgtaccaacatctactatcacgctggatctgcgcgcctcctgactgtcggtcacccatactactctattcccaagtcagacaatcccaagaaaatcgtggtacccaaagtgagcggactccagtatcgtgttttcagagtccgcttgccagatcccaacaagtttggcttcccagacacaagcttctacaatcctgaaacccaacgcctggtatgggcatgcgtgggactcgaggttggccgtggtcagcctctgggagtgggcatctcaggccacccattgctcaacaaattcgatgacaccgagaattccaacagatacgcgggtggaccaggtacagataaccgcgaatgcatcagcatggactacaagcagacccaactgtgcctcttgggctgcaagccaccaattggagagcactggggcaaaggctcaccttgctccaacaacgctatcacacctggagactgcccacccttggaactcaagaattctgtcattcaggatggtgacatggtggacactggctttggtgcaatggatttcaccgctcttcaagacaccaagtcaaacgtacctctggatatctgcaatagcatttgcaagtatccagactacctcaagatggttgctgagccttacggtgatacactgttcttctacctgagacgtgagcagatgtttgtgagacacttcttcaaccgttccggcactgtcggagagtcagttcctaacgacctctacatcaagggttctggcagcacagcaactctggcgaactcaacctactttcctactccttccggatctatggtcacgagcgatgctcagatcttcaacaagccctactggatgcaacgtgcccagggacacaacaatggcatttgctggggcaatcagctcttcgtcactgttgtggacactactcgctccactaacatgtctgtctgcgctgccattgccaactccgataccactttcaaaagctctaactttaaggaatatctgcgtcacggtgaggagttcgacttgcagttcatcttccaactctgcaagatcaccctgtccgctgatatcatgacctacattcacagcatgaatccagctatcctggaagactggaacttcggtctgaccactccaccctctggtagcctggaggatacctacaggtttgttacatctcaagcaatcacttgccagaagctgtacaagacctgcaagcaggctggtacctgccctcctgacgtgatccctaaggtggagggtccacagaagcctaaagaggaccccttcaaagattacgtcttctgggaggtgaatctgaaggagaagttctctgctgatttggatcagtttccactgggtcgtaagttcctgctccaagctggataccgtgctggtccttcgtttgccgctggcgcgggttcggctcctagcgcctcgactaccacgccggctggcggttcggccacgggcagctaag

SEQ ID NO: 48 - DNA, 1552 bp, Artificial Sequence
  gene (1)..(1552): 31L1h4428-431/dES-CS1 nt
atgagaccatcagaggctacagtatatctgccacctgttcctgtaagcaaagtggtttcaaccgatgagtacgtaacacgtaccaacatctactatcacgctggatctgcgcgcctcctgactgtcggtcacccatactactctattcccaagtcagacaatcccaagaaaatcgtggtacccaaagtgagcggactccagtatcgtgttttcagagtccgcttgccagatcccaacaagtttggcttcccagacacaagcttctacaatcctgaaacccaacgcctggtatgggcatgcgtgggactcgaggttggccgtggtcagcctctgggagtgggcatctcaggccacccattgctcaacaaattcgatgacaccgagaattccaacagatacgcgggtggaccaggtacagataaccgcgaatgcatcagcatggactacaagcagacccaactgtgcctcttgggctgcaagccaccaattggagagcactggggcaaaggctcaccttgctccaacaacgctatcacacctggagactgcccacccttggaactcaagaattctgtcattcaggatggtgacatggtggacactggctttggtgcaatggatttcaccgctcttcaagacaccaagtcaaacgtacctctggatatctgcaatagcatttgcaagtatccagactacctcaagatggttgctgagccttacggtgatacactgttcttctacctgagacgtgagcagatgtttgtgagacacttcttcaaccgttccggcactgtcggagagtcagttcctaacgacctctacatcaagggttctggcagcacagcaactctggcgaactcaacctactttcctactccttccggatctatggtcacgagcgatgctcagatcttcaacaagccctactggatgcaacgtgcccagggacacaacaatggcatttgctggggcaatcagctcttcgtcactgttgtggacactactcgctccactaacatgtctgtctgcgctgccattgccaactccgataccactttcaaaagctctaactttaaggaatatctgcgtcacggtgaggagttcgacttgcagttcatcttccaactctgcaagatcaccctgtccgctgatatcatgacctacattcacagcatgaatccagctatcctggaagactggaacttcggtctgaccactccaccctctggtagcctggaggatacctacaggtttgttacatctcaagcaatcacttgccagaagctgtacaagacctgcaagcaggctggtacctgccctcctgacgtgatccctccacagaagcctaaagaggaccccttcaaagattacgtcttctgggaggtgaatctgaaggagaagttctctgctgatttggatcagtttccactgggtcgtaagttcctgctccaagctggataccgtgctggtccttcgtttgccgctggcgcgggttcggctcctagcgcctcgactaccacgccggctggcggttcggccacgggcagctaag

SEQ ID NO: 49 - DNA, 1564 bp, Artificial Sequence
  gene (1)..(1564): 31L1h4428-431/dE-CS2 nt
atgagaccatcagaggctacagtatatctgccacctgttcctgtaagcaaagtggtttcaaccgatgagtacgtaacacgtaccaacatctactatcacgctggatctgcgcgcctcctgactgtcggtcacccatactactctattcccaagtcagacaatcccaagaaaatcgtggtacccaaagtgagcggactccagtatcgtgttttcagagtccgcttgccagatcccaacaagtttggcttcccagacacaagcttctacaatcctgaaacccaacgcctggtatgggcatgcgtgggactcgaggttggccgtggtcagcctctgggagtgggcatctcaggccacccattgctcaacaaattcgatgacaccgagaattccaacagatacgcgggtggaccaggtacagataaccgcgaatgcatcagcatggactacaagcagacccaactgtgcctcttgggctgcaagccaccaattggagagcactggggcaaaggctcaccttgctccaacaacgctatcacacctggagactgcccacccttggaactcaagaattctgtcattcaggatggtgacatggtggacactggctttggtgcaatggatttcaccgctcttcaagacaccaagtcaaacgtacctctggatatctgcaatagcatttgcaagtatccagactacctcaagatggttgctgagccttacggtgatacactgttcttctacctgagacgtgagcagatgtttgtgagacacttcttcaaccgttccggcactgtcggagagtcagttcctaacgacctctacatcaagggttctggcagcacagcaactctggcgaactcaacctactttcctactccttccggatctatggtcacgagcgatgctcagatcttcaacaagccctactggatgcaacgtgcccagggacacaacaatggcatttgctggggcaatcagctcttcgtcactgttgtggacactactcgctccactaacatgtctgtctgcgctgccattgccaactccgataccactttcaaaagctctaactttaaggaatatctgcgtcacggtgaggagttcgacttgcagttcatcttccaactctgcaagatcaccctgtccgctgatatcatgacctacattcacagcatgaatccagctatcctggaagactggaacttcggtctgaccactccaccctctggtagcctggaggatacctacaggtttgttacatctcaagcaatcacttgccagaagctgtacaagacctgcaagcaggctggtacctgccctcctgacgtgatccctaaggtggagggtccacagaagcctaaagaggaccccttcaaagattacgtcttctgggaggtgaatctgaaggagaagttctctgctgatttggatcagtttccactgggtcgtaagttcctgctccaagctggatacggcgctggtccttcgtttgccgctggcgcgggttcggctcctagcgcctcgactaccacgccggctggcggttcggccacgggcagctaag

SEQ ID NO: 50 - DNA, 1552 bp, Artificial Sequence
  gene (1)..(1552): 31L1h4428-431/dES-CS2 nt
atgagaccatcagaggctacagtatatctgccacctgttcctgtaagcaaagtggtttcaaccgatgagtacgtaacacgtaccaacatctactatcacgctggatctgcgcgcctcctgactgtcggtcacccatactactctattcccaagtcagacaatcccaagaaaatcgtggtacccaaagtgagcggactccagtatcgtgttttcagagtccgcttgccagatcccaacaagtttggcttcccagacacaagcttctacaatcctgaaacccaacgcctggtatgggcatgcgtgggactcgaggttggccgtggtcagcctctgggagtgggcatctcaggccacccattgctcaacaaattcgatgacaccgagaattccaacagatacgcgggtggaccaggtacagataaccgcgaatgcatcagcatggactacaagcagacccaactgtgcctcttgggctgcaagccaccaattggagagcactggggcaaaggctcaccttgctccaacaacgctatcacacctggagactgcccacccttggaactcaagaattctgtcattcaggatggtgacatggtggacactggctttggtgcaatggatttcaccgctcttcaagacaccaagtcaaacgtacctctggatatctgcaatagcatttgcaagtatccagactacctcaagatggttgctgagccttacggtgatacactgttcttctacctgagacgtgagcagatgtttgtgagacacttcttcaaccgttccggcactgtcggagagtcagttcctaacgacctctacatcaagggttctggcagcacagcaactctggcgaactcaacctactttcctactccttccggatctatggtcacgagcgatgctcagatcttcaacaagccctactggatgcaacgtgcccagggacacaacaatggcatttgctggggcaatcagctcttcgtcactgttgtggacactactcgctccactaacatgtctgtctgcgctgccattgccaactccgataccactttcaaaagctctaactttaaggaatatctgcgtcacggtgaggagttcgacttgcagttcatcttccaactctgcaagatcaccctgtccgctgatatcatgacctacattcacagcatgaatccagctatcctggaagactggaacttcggtctgaccactccaccctctggtagcctggaggatacctacaggtttgttacatctcaagcaatcacttgccagaagctgtacaagacctgcaagcaggctggtacctgccctcctgacgtgatccctccacagaagcctaaagaggaccccttcaaagattacgtcttctgggaggtgaatctgaaggagaagttctctgctgatttggatcagtttccactgggtcgtaagttcctgctccaagctggatacggcgctggtccttcgtttgccgctggcgcgggttcggctcctagcgcctcgactaccacgccggctggcggttcggccacgggcagctaag

SEQ ID NO: 51 - DNA, 1564 bp, Artificial Sequence
  gene (1)..(1564): 31L1h4428-431/dE-CS3 nt
atgagaccatcagaggctacagtatatctgccacctgttcctgtaagcaaagtggtttcaaccgatgagtacgtaacacgtaccaacatctactatcacgctggatctgcgcgcctcctgactgtcggtcacccatactactctattcccaagtcagacaatcccaagaaaatcgtggtacccaaagtgagcggactccagtatcgtgttttcagagtccgcttgccagatcccaacaagtttggcttcccagacacaagcttctacaatcctgaaacccaacgcctggtatgggcatgcgtgggactcgaggttggccgtggtcagcctctgggagtgggcatctcaggccacccattgctcaacaaattcgatgacaccgagaattccaacagatacgcgggtggaccaggtacagataaccgcgaatgcatcagcatggactacaagcagacccaactgtgcctcttgggctgcaagccaccaattggagagcactggggcaaaggctcaccttgctccaacaacgctatcacacctggagactgcccacccttggaactcaagaattctgtcattcaggatggtgacatggtggacactggctttggtgcaatggatttcaccgctcttcaagacaccaagtcaaacgtacctctggatatctgcaatagcatttgcaagtatccagactacctcaagatggttgctgagccttacggtgatacactgttcttctacctgagacgtgagcagatgtttgtgagacacttcttcaaccgttccggcactgtcggagagtcagttcctaacgacctctacatcaagggttctggcagcacagcaactctggcgaactcaacctactttcctactccttccggatctatggtcacgagcgatgctcagatcttcaacaagccctactggatgcaacgtgcccagggacacaacaatggcatttgctggggcaatcagctcttcgtcactgttgtggacactactcgctccactaacatgtctgtctgcgctgccattgccaactccgataccactttcaaaagctctaactttaaggaatatctgcgtcacggtgaggagttcgacttgcagttcatcttccaactctgcaagatcaccctgtccgctgatatcatgacctacattcacagcatgaatccagctatcctggaagactggaacttcggtctgaccactccaccctctggtagcctggaggatacctacaggtttgttacatctcaagcaatcacttgccagaagctgtacaagacctgcaagcaggctggtacctgccctcctgacgtgatccctaaggtggagggtccacagaagcctaaagaggaccccttcaaagattacgtcttctgggaggtgaatctgaaggagaagttctctgctgatttggatcagtttccactgggtcgtaagttcctgctccaagctggataccgtgctggtccttcgtttaaagctggcgcgggttcggctcctagcgcctcgactaccacgccggctggcggttcggccacgggcagctaag

SEQ ID NO: 52 - DNA, 1552 bp, Artificial Sequence
  gene (1)..(1552): 31L1h4428-431/dES-CS3 nt
atgagaccatcagaggctacagtatatctgccacctgttcctgtaagcaaagtggtttcaaccgatgagtacgtaacacgtaccaacatctactatcacgctggatctgcgcgcctcctgactgtcggtcacccatactactctattcccaagtcagacaatcccaagaaaatcgtggtacccaaagtgagcggactccagtatcgtgttttcagagtccgcttgccagatcccaacaagtttggcttcccagacacaagcttctacaatcctgaaacccaacgcctggtatgggcatgcgtgggactcgaggttggccgtggtcagcctctgggagtgggcatctcaggccacccattgctcaacaaattcgatgacaccgagaattccaacagatacgcgggtggaccaggtacagataaccgcgaatgcatcagcatggactacaagcagacccaactgtgcctcttgggctgcaagccaccaattggagagcactggggcaaaggctcaccttgctccaacaacgctatcacacctggagactgcccacccttggaactcaagaattctgtcattcaggatggtgacatggtggacactggctttggtgcaatggatttcaccgctcttcaagacaccaagtcaaacgtacctctggatatctgcaatagcatttgcaagtatccagactacctcaagatggttgctgagccttacggtgatacactgttcttctacctgagacgtgagcagatgtttgtgagacacttcttcaaccgttccggcactgtcggagagtcagttcctaacgacctctacatcaagggttctggcagcacagcaactctggcgaactcaacctactttcctactccttccggatctatggtcacgagcgatgctcagatcttcaacaagccctactggatgcaacgtgcccagggacacaacaatggcatttgctggggcaatcagctcttcgtcactgttgtggacactactcgctccactaacatgtctgtctgcgctgccattgccaactccgataccactttcaaaagctctaactttaaggaatatctgcgtcacggtgaggagttcgacttgcagttcatcttccaactctgcaagatcaccctgtccgctgatatcatgacctacattcacagcatgaatccagctatcctggaagactggaacttcggtctgaccactccaccctctggtagcctggaggatacctacaggtttgttacatctcaagcaatcacttgccagaagctgtacaagacctgcaagcaggctggtacctgccctcctgacgtgatccctccacagaagcctaaagaggaccccttcaaagattacgtcttctgggaggtgaatctgaaggagaagttctctgctgatttggatcagtttccactgggtcgtaagttcctgctccaagctggataccgtgctggtccttcgtttaaagctggcgcgggttcggctcctagcgcctcgactaccacgccggctggcggttcggccacgggcagctaag

SEQ ID NO: 53 - protein, 23 aa, HPV35
TQLYRTCKAAGTCPPDVIPKVEG

SEQ ID NO: 54 - protein, 23 aa, HPV39
STLYRTCKQSGTCPPDVVDKVEG

SEQ ID NO: 55 - protein, 23 aa, HPV51
TQLYSTCKAAGTCPPDVVNKVEG

SEQ ID NO: 56 - protein, 23 aa, HPV53
TQLYQTCKQSGTCPEDVINKIEH

SEQ ID NO: 57 - protein, 23 aa, HPV56
TQLYKTCKLSGTCPEDVVNKIEQ

SEQ ID NO: 58 - protein, 23 aa, HPV68
STLYKTCKQSGTCPPDVINKVEG

SEQ ID NO: 59 - protein, 23 aa, HPV73
TQLYKTCKQAGTCPPDVIPKVEG

SEQ ID NO: 60 - protein, 23 aa, HPV82
TQLYSTCKAAGTCPPDVIPKVKG